European Patent Application EP 4 434 517 A1, published September 25, 2024. Title: 一种抗SOST抗体药物组合物及其用途. Applicant: 江苏恒瑞医药股份有限公司. Application CN. The sequence listing filed with the application follows.

SEQUENCE LISTING (27 sequences)

SEQ ID NO: 1 - protein, 117 aa, Mus musculus
EVQLQQSGPELVKPGTSVKIPCQTSGYTFTDYNLDWLKQRPGESLEWIGDIDPNNGDILYNQKFRDKATLTVDTSSNTAYLELRSLTSEDTAVYYCARRWAYYFDYWGQGTTLTISS

SEQ ID NO: 2 - protein, 107 aa, Mus musculus
NIVMTQTPKLLFVSAGDRITITCKASQSVSNDVAWYQQKPGQSPKLLIYYTSNRFTGVPDRFTGSGYGTDFTLTINTVQAEDLAVYFCQQDYSSPVTFGAGTKLELK

SEQ ID NO: 3 - protein, 5 aa, Mus musculus
DYNLD

SEQ ID NO: 4 - protein, 17 aa, Mus musculus
DIDPNNGDILYNQKFRD

SEQ ID NO: 5 - protein, 8 aa, Mus musculus
RWAYYFDY

SEQ ID NO: 6 - protein, 11 aa, Mus musculus
KASQSVSNDVA

SEQ ID NO: 7 - protein, 7 aa, Mus musculus
YTSNRFT

SEQ ID NO: 8 - protein, 9 aa, Mus musculus
QQDYSSPVT

SEQ ID NO: 9 - protein, 17 aa, synthetic construct
  REGION 1..17: note = Ab-1CDR2
DIDPNDGDILYNQKFRD

SEQ ID NO: 10 - protein, 117 aa, synthetic construct
  REGION 1..117: note = Ab-5
EVQLVQSGAEVKKPGASVKVSCKASGYTFTDYNLDWLRQAPGEGLEWIGDIDPNDGDILYNQKFRDRVTMTTDTSTSTAYMELRSLRSDDTAVYYCARRWAYYFDYWGQGTTVTVSS

SEQ ID NO: 11 - protein, 117 aa, synthetic construct
  REGION 1..117: note = Ab-9
EVQLVQSGAEVKKPGASVKVSCKASGYTFTDYNLDWLRQAPGEGLEWIGDIDPNNGDILYNQKFRDRVTMTTDTSTSTAYMELRSLRSDDTAVYYCARRWAYYFDYWGQGTTVTVSS

SEQ ID NO: 12 - protein, 117 aa, synthetic construct
  REGION 1..117: note = Ab-10
EVQLVQSGAEVKKPGASVKVSCKASGYTFTDYNLDWVRQAPGQGLEWMGDIDPNNGDILYNQKFRDRVTMTTDTSTSTAYMELRSLRSDDTAVYYCARRWAYYFDYWGQGTTVTVSS

SEQ ID NO: 13 - protein, 107 aa, synthetic construct
  REGION 1..107: note = Ab-5
DIVMTQSPSSLSASVGDRVTITCKASQSVSNDVAWYQQKPGKSPKLLIYYTSNRFTGVPDRFSGSGSGTDFTLTISSLQPEDFATYFCQQDYSSPVTFGGGTKVEIK

SEQ ID NO: 14 - protein, 107 aa, synthetic construct
  REGION 1..107: note = Ab-9
NIVMTQSPSSLSASVGDRVTITCKASQSVSNDVAWYQQKPGKSPKLLIYYTSNRFTGVPDRFSGSGSGTDFTLTISSLQPEDFATYFCQQDYSSPVTFGGGTKVEIK

SEQ ID NO: 15 - protein, 107 aa, synthetic construct
  REGION 1..107: note = Ab-10
DIQMTQSPSSLSASVGDRVTITCKASQSVSNDVAWYQQKPGKAPKLLIYYTSNRFTGVPSRFSGSGSGTDFTLTISSLQPEDFATYYCQQDYSSPVTFGGGTKVEIK

SEQ ID NO: 16 - protein, 326 aa, synthetic construct
  REGION 1..326: note = CKIgG4
ASTKGPSVFPLAPCSRSTSESTAALGCLVKDYFPEPVTVSWNSGALTSGVHTFPAVLQSSGLYSLSSVVTVPSSSLGTKTYTCNVDHKPSNTKVDKRVESKYGPPCPPCPAPEFLGGPSVFLFPPKPKDTLMISRTPEVTCVVVDVSQEDPEVQFNWYVDGVEVHNAKTKPREEQFNSTYRVVSVLTVLHQDWLNGKEYKCKVSNKGLPSSIEKTISKAKGQPREPQVYTLPPSQEEMTKNQVSLTCLVKGFYPSDIAVEWESNGQPENNYKTTPPVLDSDGSFFLYSRLTVDKSRWQEGNVFSCSVMHEALHNHYTQKSLSLSLG

SEQ ID NO: 17 - protein, 327 aa, synthetic construct
  REGION 1..327: note = IgG4
ASTKGPSVFPLAPCSRSTSESTAALGCLVKDYFPEPVTVSWNSGALTSGVHTFPAVLQSSGLYSLSSVVTVPSSSLGTKTYTCNVDHKPSNTKVDKRVESKYGPPCPPCPAPEFLGGPSVFLFPPKPKDTLMISRTPEVTCVVVDVSQEDPEVQFNWYVDGVEVHNAKTKPREEQFNSTYRVVSVLTVLHQDWLNGKEYKCKVSNKGLPSSIEKTISKAKGQPREPQVYTLPPSQEEMTKNQVSLTCLVKGFYPSDIAVEWESNGQPENNYKTTPPVLDSDGSFFLYSRLTVDKSRWQEGNVFSCSVMHEALHNHYTQKSLSLSLGK

SEQ ID NO: 18 - protein, 330 aa, synthetic construct [sequence omitted]

SEQ ID NO: 19 - protein, 107 aa, synthetic construct [sequence omitted]

SEQ ID NO: 20 - protein, 447 aa, synthetic construct
  REGION 1..447: note = Ab-10
EVQLVQSGAEVKKPGASVKVSCKASGYTFTDYNLDWVRQAPGQGLEWMGDIDPNNGDILYNQKFRDRVTMTTDTSTSTAYMELRSLRSDDTAVYYCARRWAYYFDYWGQGTTVTVSSASTKGPSVFPLAPSSKSTSGGTAALGCLVKDYFPEPVTVSWNSGALTSGVHTFPAVLQSSGLYSLSSVVTVPSSSLGTQTYICNVNHKPSNTKVDKKVEPKSCDKTHTCPPCPAPELLGGPSVFLFPPKPKDTLMISRTPEVTCVVVDVSHEDPEVKFNWYVDGVEVHNAKTKPREEQYNSTYRVVSVLTVLHQDWLNGKEYKCKVSNKALPAPIEKTISKAKGQPREPQVYTLPPSRDELTKNQVSLTCLVKGFYPSDIAVEWESNGQPENNYKTTPPVLDSDGSFFLYSKLTVDKSRWQQGNVFSCSVMHEALHNHYTQKSLSLSPGK

SEQ ID NO: 21 - protein, 444 aa, synthetic construct
  REGION 1..444: note = Ab-9
EVQLVQSGAEVKKPGASVKVSCKASGYTFTDYNLDWLRQAPGEGLEWIGDIDPNNGDILYNQKFRDRVTMTTDTSTSTAYMELRSLRSDDTAVYYCARRWAYYFDYWGQGTTVTVSSASTKGPSVFPLAPCSRSTSESTAALGCLVKDYFPEPVTVSWNSGALTSGVHTFPAVLQSSGLYSLSSVVTVPSSSLGTKTYTCNVDHKPSNTKVDKRVESKYGPPCPPCPAPEFLGGPSVFLFPPKPKDTLMISRTPEVTCVVVDVSQEDPEVQFNWYVDGVEVHNAKTKPREEQFNSTYRVVSVLTVLHQDWLNGKEYKCKVSNKGLPSSIEKTISKAKGQPREPQVYTLPPSQEEMTKNQVSLTCLVKGFYPSDIAVEWESNGQPENNYKTTPPVLDSDGSFFLYSRLTVDKSRWQEGNVFSCSVMHEALHNHYTQKSLSLSLGK

SEQ ID NO: 22 - protein, 443 aa, synthetic construct
  REGION 1..443: note = Ab-5
EVQLVQSGAEVKKPGASVKVSCKASGYTFTDYNLDWLRQAPGEGLEWIGDIDPNDGDILYNQKFRDRVTMTTDTSTSTAYMELRSLRSDDTAVYYCARRWAYYFDYWGQGTTVTVSSASTKGPSVFPLAPCSRSTSESTAALGCLVKDYFPEPVTVSWNSGALTSGVHTFPAVLQSSGLYSLSSVVTVPSSSLGTKTYTCNVDHKPSNTKVDKRVESKYGPPCPPCPAPEFLGGPSVFLFPPKPKDTLMISRTPEVTCVVVDVSQEDPEVQFNWYVDGVEVHNAKTKPREEQFNSTYRVVSVLTVLHQDWLNGKEYKCKVSNKGLPSSIEKTISKAKGQPREPQVYTLPPSQEEMTKNQVSLTCLVKGFYPSDIAVEWESNGQPENNYKTTPPVLDSDGSFFLYSRLTVDKSRWQEGNVFSCSVMHEALHNHYTQKSLSLSLG

SEQ ID NO: 23 - protein, 214 aa, synthetic construct
  REGION 1..214: note = Ab-10
DIQMTQSPSSLSASVGDRVTITCKASQSVSNDVAWYQQKPGKAPKLLIYYTSNRFTGVPSRFSGSGSGTDFTLTISSLQPEDFATYYCQQDYSSPVTFGGGTKVEIKRTVAAPSVFIFPPSDEQLKSGTASVVCLLNNFYPREAKVQWKVDNALQSGNSQESVTEQDSKDSTYSLSSTLTLSKADYEKHKVYACEVTHQGLSSPVTKSFNRGEC

SEQ ID NO: 24 - protein, 214 aa, synthetic construct
  REGION 1..214: note = Ab-9
NIVMTQSPSSLSASVGDRVTITCKASQSVSNDVAWYQQKPGKSPKLLIYYTSNRFTGVPDRFSGSGSGTDFTLTISSLQPEDFATYFCQQDYSSPVTFGGGTKVEIKRTVAAPSVFIFPPSDEQLKSGTASVVCLLNNFYPREAKVQWKVDNALQSGNSQESVTEQDSKDSTYSLSSTLTLSKADYEKHKVYACEVTHQGLSSPVTKSFNRGEC

SEQ ID NO: 25 - protein, 214 aa, synthetic construct
  REGION 1..214: note = Ab-5
DIVMTQSPSSLSASVGDRVTITCKASQSVSNDVAWYQQKPGKSPKLLIYYTSNRFTGVPDRFSGSGSGTDFTLTISSLQPEDFATYFCQQDYSSPVTFGGGTKVEIKRTVAAPSVFIFPPSDEQLKSGTASVVCLLNNFYPREAKVQWKVDNALQSGNSQESVTEQDSKDSTYSLSSTLTLSKADYEKHKVYACEVTHQGLSSPVTKSFNRGEC

SEQ ID NO: 26 - protein, 101 aa, synthetic construct
  REGION 1..101: note = H1
EVQLVQSGAEVKKPGASVKVSCKASGYTFTDYNLDWLRQAPGEGLEWIGDIDPNDGDILYNQKFRDRVTMTTDTSTSTAYMELRSLRSDDTAVYYCARRWA

SEQ ID NO: 27 - protein, 341 aa, synthetic construct
  REGION 1..341: note = H2
YFDYWGQGTTVTVSSASTKGPSVFPLAPCSRSTSESTAALGCLVKDYFPEPVTVSWNSGALTSGVHTFPAVLQSSGLYSLSSVVTVPSSSLGTKTYTCNVDHKPSNTKVDKRVESKYGPPCPPCPAPEFLGGPSVFLFPPKPKDTLMISRTPEVTCVVVDVSQEDPEVQFNWYVDGVEVHNAKTKPREEQFNSTYRVVSVLTVLHQDWLNGKEYKCKVSNKGLPSSIEKTISKAKGQPREPQVYTLPPSQEEMTKNQVSLTCLVKGFYPSDIAVEWESNGQPENNYKTTPPVLDSDGSFFLYSRLTVDKSRWQEGNVFSCSVMHEALHNHYTQKSLSLSLG